European Patent Application EP 4 230 645 A1, published August 23, 2023. Title: Peptidic inhibitors of amyloid self- and cross-assembly. Applicant: Technische Universitaet Muenchen. The sequence listing filed with the application follows.

SEQUENCE LISTING (48 sequences)

SEQ ID NO: 1 - protein, 26 aa, Artificial Sequence
  Formula 1
  VARIANT 1: selected from glutamine, asparagine, alanine, glutamic acid, and aspartic acid, preferably is glutamine
  VARIANT 1,2,3,4,24,25,26: optionally present
  VARIANT 2: selected from lysine, modified lysine e.g. Lys(Ac), Lys(N3), and Lys(biotin), alanine, modified alanine, ornithine, modified ornit hine e.g. Orn(Ac), diaminobutyric acid, diaminopropionic acid, ar ginine, and modified arginine e.g. Arg(Me)2, preferably is lysine
  VARIANT 3: selected from leucine, N-methyl-leucine, alanine, N-methyl-alanin e, isoleucine, N-methyl-isoleucine, valine, N-methyl-valine, glyc ine, N-methyl-glycine, norleucine, N-methyl-norleucine, phenylala nine, N-methyl-phenylalanine, tyrosine, and N-methyl-tyrosine, preferably is leucine or N-methyl-leucine
  VARIANT 4: selected from leucine, N-methyl-leucine, alanine, N-methyl-alanin e, isoleucine, N-methyl-isoleucine, valine, N-methyl-valine, glyc ine, N-methyl-glycine, norleucine, N-methyl-norleucine, phenylala nine, N-methyl-phenylalanine, tyrosine, and N-methyl-tyrosine, preferably is valine or N-methyl-valine
  VARIANT 5,6: selected from phenylalanine, N-methyl-phenylalanine, halogenated phenylalanine, tyrosine, and N-methyl-tyrosine, preferably selected from phenylalanine and N-methyl-phenylalanine
  VARIANT 7,16: selected from alanine, N-methyl-alanine, leucine, N-methyl-leucine, valine, N-methyl-valine, glycine, and N-methyl-glycine, preferably is alanine
  VARIANT 8: selected from glutamic acid, N-methyl-glutamic acid, aspartic acid, N-methyl-aspartic acid, glutamine, N-methyl-glutamine, asparagine, N-methyl-asparagine, alanine, N-methyl-alanine, glycine, and N-methyl-glycine, preferably is glutamic acid
  VARIANT 9: selected from aspartic acid, glutamic acid, asparagine, aspartic acid, alanine, and glycine, preferably is aspartic acid
  VARIANT 10,11,12: selected from norleucine, leucine, phenylalanine, methionine, tryptophan, tyrosine, threonine, alanine, isoleucine, valine, and modified forms thereof e.g. N-methylated forms thereof, preferably selected from norleucine, leucine, and phenylalanine
  VARIANT 13: selected from asparagine, glutamine and alanine, preferably is asparagine
  VARIANT 14: selected from lysine, modified lysine e.g. Lys(Ac), Lys(N3), and Lys(biotin), alanine, norleucine, ornithine, modified ornithine e .g. Orn(Ac), diaminobutyric acid, diaminopropionic acid, arginine , and modified arginine e.g. Arg(Me)2, preferably is lysine
  VARIANT 15,23,24: selected from glycine and alanine, preferably is glycine
  VARIANT 17,18: selected from isoleucine, leucine, norleucine, and valine, preferably is isoleucine
  VARIANT 19: selected from glycine, alanine, and serine, preferably is glycine
  VARIANT 20: selected from leucine, alanine, isoleucine, threonine, norleucine, and valine, preferably is leucine
  VARIANT 21: selected from norleucine, leucine, phenylalanine, methionine, tryptophan, tyrosine, threonine, alanine, isoleucine, and valine, preferably is norleucine
XXXXFFAEXXXXNKGAIIXXXVGGVV

SEQ ID NO: 2 - protein, 26 aa, Artificial Sequence
  formula 2
  VARIANT 1: selected from glutamine, asparagine, alanine, glutamic acid, and aspartic acid, preferably is glutamine
  VARIANT 1,2,3,4,24,25,26: optionally present
  VARIANT 2: selected from lysine, modified lysine e.g. Lys(Ac), Lys(N3), and Lys(biotin), alanine, modified alanine, ornithine, modified ornit hine e.g. Orn(Ac), diaminobutyric acid, diaminopropionic acid, ar ginine, and modified arginine e.g. Arg(Me)2, preferably is lysine
  VARIANT 3: leucine or N-methyl-leucine
  VARIANT 4: valine or N-methyl-valine
  VARIANT 5,6: selected from phenylalanine, N-methyl-phenylalanine, halogenated phenylalanine, tyrosine, and N-methyl-tyrosine, preferably selected from phenylalanine and N-methyl-phenylalanine
  VARIANT 7,16: selected from alanine, N-methyl-alanine, leucine, N-methyl-leucine, valine, N-methyl-valine, glycine, and N-methyl-glycine, preferably is alanine
  VARIANT 8: selected from glutamic acid, N-methyl-glutamic acid, aspartic acid, N-methyl-aspartic acid, glutamine, N-methyl-glutamine, asparagine, N-methyl-asparagine, alanine, N-methyl-alanine, glycine, and N-methyl-glycine, preferably is glutamic acid
  VARIANT 9: selected from aspartic acid, glutamic acid, asparagine, aspartic acid, alanine, and glycine, preferably is aspartic acid
  VARIANT 10,11,12: selected from norleucine, leucine, phenylalanine, methionine, tryptophan, tyrosine, threonine, alanine, isoleucine, valine, and modified forms thereof e.g. N-methylated forms thereof, preferably selected from norleucine, leucine, and phenylalanine
  VARIANT 13: selected from asparagine, glutamine and alanine, preferably is asparagine
  VARIANT 14: selected from lysine, modified lysine e.g. Lys(Ac), Lys(N3), and Lys(biotin), alanine, norleucine, ornithine, modified ornithine e .g. Orn(Ac), diaminobutyric acid, diaminopropionic acid, arginine , and modified arginine e.g. Arg(Me)2, preferably is lysine
  VARIANT 15,23,24: selected from glycine and alanine, preferably is glycine
  VARIANT 17,18: selected from isoleucine, leucine, norleucine, and valine, preferably is isoleucine
  VARIANT 19: selected from glycine, alanine, and serine, preferably is glycine
  VARIANT 20: selected from leucine, alanine, isoleucine, threonine, norleucine, and valine, preferably is leucine
  VARIANT 21: selected from norleucine, leucine, phenylalanine, methionine, tryptophan, tyrosine, threonine, alanine, isoleucine, and valine, preferably is norleucine
XXLVFFAEXXXXNKGAIIXXXVGGVV

SEQ ID NO: 3 - protein, 26 aa, Artificial Sequence
  formula 3
  VARIANT 3: leucine or N-methyl-leucine
  VARIANT 4: valine or N-methyl-valine
  VARIANT 5,6: phenylalanine or N-methyl-phenylalanine
  VARIANT 10,11,12: selected from norleucine, leucine, phenylalanine, methionine, tryptophan, tyrosine, threonine, alanine, isoleucine, and valine, preferably selected from norleucine, leucine, and phenylalanine
  VARIANT 21: norleucine
QKLVFFAEDXXXNKGAIIGLXVGGVV

SEQ ID NO: 4 - protein, 22 aa, Artificial Sequence
  formula 4
  VARIANT 1,2: phenylalanine or N-methyl-phenylalanine
  VARIANT 6,7,8: selected from norleucine, leucine, phenylalanine, methionine, tryptophan, tyrosine, threonine, alanine, isoleucine, and valine, preferably selected from norleucine, leucine, and phenylalanine
  VARIANT 17: norleucine
FFAEDXXXNKGAIIGLXVGGVV

SEQ ID NO: 5 - protein, 23 aa, Artificial Sequence
  formula 5
  VARIANT 3: leucine or N-methyl-leucine
  VARIANT 4: valine or N-methyl-valine
  VARIANT 5,6: phenylalanine or N-methyl-phenylalanine
  VARIANT 10,11,12: selected from norleucine, leucine, phenylalanine, methionine, tryptophan, tyrosine, threonine, alanine, isoleucine, and valine, preferably selected from norleucine, leucine, and phenylalanine
  VARIANT 21: norleucine
QKLVFFAEDXXXNKGAIIGLXVG

SEQ ID NO: 6 - protein, 26 aa, Artificial Sequence
  formula 6
  VARIANT 3: leucine or N-methyl-leucine
  VARIANT 4: valine or N-methyl-valine
  VARIANT 5,6: phenylalanine or N-methyl-phenylalanine
  VARIANT 10,11,12,21: norleucine
QKLVFFAEDXXXNKGAIIGLXVGGVV

SEQ ID NO: 7 - protein, 26 aa, Artificial Sequence
  formula 7
  VARIANT 3: leucine or N-methyl-leucine
  VARIANT 4: valine or N-methyl-valine
  VARIANT 5,6: phenylalanine or N-methyl-phenylalanine
  VARIANT 21: norleucine
QKLVFFAEDLLLNKGAIIGLXVGGVV

SEQ ID NO: 8 - protein, 26 aa, Artificial Sequence
  formula 8
  VARIANT 3: leucine or N-methyl-leucine
  VARIANT 4: valine or N-methyl-valine
  VARIANT 5,6: phenylalanine or N-methyl-phenylalanine
  VARIANT 21: norleucine
QKLVFFAEDFFFNKGAIIGLXVGGVV

SEQ ID NO: 9 - protein, 26 aa, Artificial Sequence
  formula 9
  VARIANT 3,5: N-methylated
  VARIANT 10,11,12,21: norleucine
QKLVFFAEDXXXNKGAIIGLXVGGVV

SEQ ID NO: 10 - protein, 26 aa, Artificial Sequence
  formula 10
  VARIANT 4,6: N-methylated
  VARIANT 10,11,12,21: norleucine
QKLVFFAEDXXXNKGAIIGLXVGGVV

SEQ ID NO: 11 - protein, 26 aa, Artificial Sequence
  formula 11
  VARIANT 3,5: N-methylated
  VARIANT 21: norleucine
QKLVFFAEDLLLNKGAIIGLXVGGVV

SEQ ID NO: 12 - protein, 26 aa, Artificial Sequence
  formula 12
  VARIANT 4,6: N-methylated
  VARIANT 21: norleucine
QKLVFFAEDLLLNKGAIIGLXVGGVV

SEQ ID NO: 13 - protein, 26 aa, Artificial Sequence
  formula 13
  VARIANT 3,5: N-methylated
  VARIANT 21: norleucine
QKLVFFAEDFFFNKGAIIGLXVGGVV

SEQ ID NO: 14 - protein, 26 aa, Artificial Sequence
  formula 14
  VARIANT 4,6: N-methylated
  VARIANT 21: norleucine
QKLVFFAEDFFFNKGAIIGLXVGGVV

SEQ ID NO: 15 - protein, 26 aa, Artificial Sequence
  formula 15
  VARIANT 3,4,5,6: N-methylated
  VARIANT 21: norleucine
QKLVFFAEDFFFNKGAIIGLXVGGVV

SEQ ID NO: 16 - protein, 26 aa, Artificial Sequence
  formula 16
  VARIANT 3,4,5,6: N-methylated
  VARIANT 21: norleucine
QKLVFFAEDLLLNKGAIIGLXVGGVV

SEQ ID NO: 17 - protein, 26 aa, Artificial Sequence
  formula 17
  VARIANT 3,4,5,6: N-methylated
  VARIANT 10,11,12,21: norleucine
QKLVFFAEDXXXNKGAIIGLXVGGVV

SEQ ID NO: 18 - protein, 4 aa, Artificial Sequence
  Hot sequence
  VARIANT 1,2: selected from phenylalanine, N-methyl-phenylalanine, halogenated phenylalanine, tyrosine, and N-methyl-tyrosine, preferably selected from phenylalanine and N-methyl-phenylalanine
FFAE

SEQ ID NO: 19 - protein, 6 aa, Artificial Sequence
  Hot sequence
NKGAII

SEQ ID NO: 20 - protein, 5 aa, Artificial Sequence
  Hot sequence
VGGVV

SEQ ID NO: 21 - protein, 4 aa, Artificial Sequence
  N-terminal segment
QKLV

SEQ ID NO: 22 - protein, 5 aa, Artificial Sequence
  N-terminal segment
QKLVF

SEQ ID NO: 23 - protein, 6 aa, Artificial Sequence
  N-terminal segment
QKLVFF

SEQ ID NO: 24 - protein, 4 aa, Artificial Sequence
  C-terminal segment
GGVV

SEQ ID NO: 25 - protein, 26 aa, Homo sapiens
  Abeta (15-40)
QKLVFFAEDVGSNKGAIIGLMVGGVV

SEQ ID NO: 26 - protein, 26 aa, Artificial Sequence
  Nle3
  VARIANT 10,11,12,21: norleucine
QKLVFFAEDXXXNKGAIIGLXVGGVV

SEQ ID NO: 27 - protein, 26 aa, Artificial Sequence
  Nle3-VF
  VARIANT 4,6: N-methylated
  VARIANT 10,11,12,21: norleucine
QKLVFFAEDXXXNKGAIIGLXVGGVV

SEQ ID NO: 28 - protein, 26 aa, Artificial Sequence
  Nle3-LF
  VARIANT 3,5: N-methylated
  VARIANT 10,11,12,21: norleucine
QKLVFFAEDXXXNKGAIIGLXVGGVV

SEQ ID NO: 29 - protein, 26 aa, Artificial Sequence
  Nle3-GI
  VARIANT 10,11,12,21: norleucine
  VARIANT 15,17: N-methylated
QKLVFFAEDXXXNKGAIIGLXVGGVV

SEQ ID NO: 30 - protein, 26 aa, Artificial Sequence
  Nle3-GG
  VARIANT 10,11,12,21: norleucine
  VARIANT 15,19: N-methylated
QKLVFFAEDXXXNKGAIIGLXVGGVV

SEQ ID NO: 31 - protein, 26 aa, Artificial Sequence
  L3
  VARIANT 21: norleucine
QKLVFFAEDLLLNKGAIIGLXVGGVV

SEQ ID NO: 32 - protein, 26 aa, Artificial Sequence
  L3-VF
  VARIANT 4,6: N-methylated
  VARIANT 21: norleucine
QKLVFFAEDLLLNKGAIIGLXVGGVV

SEQ ID NO: 33 - protein, 26 aa, Artificial Sequence
  L3-LF
  VARIANT 3,5: N-methylated
  VARIANT 21: norleucine
QKLVFFAEDLLLNKGAIIGLXVGGVV

SEQ ID NO: 34 - protein, 26 aa, Artificial Sequence
  F3-VF
  VARIANT 4,6: N-methylated
  VARIANT 21: norleucine
QKLVFFAEDFFFNKGAIIGLXVGGVV

SEQ ID NO: 35 - protein, 26 aa, Artificial Sequence
  F3-LF
  VARIANT 3,5: N-methylated
  VARIANT 21: norleucine
QKLVFFAEDFFFNKGAIIGLXVGGVV

SEQ ID NO: 36 - protein, 26 aa, Artificial Sequence
  VGS (Abeta (15-40))
  VARIANT 21: norleucine
QKLVFFAEDVGSNKGAIIGLXVGGVV

SEQ ID NO: 37 - protein, 26 aa, Artificial Sequence
  VGS-VF
  VARIANT 4,6: N-methylated
  VARIANT 21: norleucine
QKLVFFAEDVGSNKGAIIGLXVGGVV

SEQ ID NO: 38 - protein, 26 aa, Artificial Sequence
  VGS-LF
  VARIANT 3,5: N-methylated
  VARIANT 21: norleucine
QKLVFFAEDVGSNKGAIIGLXVGGVV

SEQ ID NO: 39 - protein, 26 aa, Artificial Sequence
  R3
  VARIANT 21: norleucine
QKLVFFAEDRRRNKGAIIGLXVGGVV

SEQ ID NO: 40 - protein, 26 aa, Artificial Sequence
  R3-VF
  VARIANT 4,6: N-methylated
  VARIANT 21: norleucine
QKLVFFAEDRRRNKGAIIGLXVGGVV

SEQ ID NO: 41 - protein, 26 aa, Artificial Sequence
  R3-LF
  VARIANT 3,5: N-methylated
  VARIANT 21: norleucine
QKLVFFAEDRRRNKGAIIGLXVGGVV

SEQ ID NO: 42 - protein, 26 aa, Artificial Sequence
  G3
  VARIANT 21: norleucine
QKLVFFAEDGGGNKGAIIGLXVGGVV

SEQ ID NO: 43 - protein, 26 aa, Artificial Sequence
  G3-VF
  VARIANT 4,6: N-methylated
  VARIANT 21: norleucine
QKLVFFAEDGGGNKGAIIGLXVGGVV

SEQ ID NO: 44 - protein, 37 aa, Homo sapiens [sequence omitted]

SEQ ID NO: 45 - protein, 42 aa, Homo sapiens [sequence omitted]

SEQ ID NO: 46 - protein, 9 aa, Artificial Sequence
  Nle3-VF (15-23)
  VARIANT 4,6: N-methylated
QKLVFFAED

SEQ ID NO: 47 - protein, 14 aa, Artificial Sequence
  Nle3-VF (27-40)
  VARIANT 9: norleucine
NKGAIIGLXVGGVV

SEQ ID NO: 48 - protein, 20 aa, Artificial Sequence
  Nle3-VF (21-40)
  VARIANT 4,5,6,15: norleucine
AEDXXXNKGAIIGLXVGGVV